European Patent Specification EP 3 142 673 B1, published September 9, 2026. Title: IMPROVED POLYETHYLENEIMINE POLYETHYLENEGLYCOL VECTORS. Applicant: Alex Levitzki management and holdings, Ltd Levitzki, Alexander Joubran, Salim Shir, Alexei Zigler, Maya. The sequence listing filed with the application follows.

SEQUENCE LISTING (6 sequences)

SEQ ID NO: 1 - protein, 12 aa, Artificial Sequence
  Synthetic
YHWYGYTPQNVI

SEQ ID NO: 2 - protein, 7 aa, Artificial Sequence
  Synthetic
  X is 8-aminooctanoic acid. (1)..(1)
XFGWWGC

SEQ ID NO: 3 - protein, 6 aa, Artificial Sequence
  Synthetic
  X is 8-aminooctanoic acid (1)..(1)
  X is diaminopropionic acid (4)..(4)
XFFXDC

SEQ ID NO: 4 - protein, 82 aa, Artificial Sequence
  Synthetic
MGSSHHHHHHSSGLVPRGSHMASAEAKYAKEMWAAWEEIRNLPNLTGWQMTAFIAKLVDDPSQSSELLSEAKKLNDSQAPKC

SEQ ID NO: 5 - protein, 79 aa, Artificial Sequence
  Synthetic
MGSSHHHHHHSSGLVPRGSHMAEAKYAKMRNAYWEIALLPNLTNQQKRAFIRKLYDDPSQSSELLSEAKKLNDSQAPKC

SEQ ID NO: 6 - protein, 53 aa, Homo sapiens
NSDSECPLSHDGYCLHDGVCMYIEALDKYACNCVVGYIGERCQYRDLKWWELR